European Patent Specification EP 3 901 278 B1, published October 23, 2024. Title: ALLELE-SPECIFIC AMPLIFICATION USING A COMPOSITION OF OVERLAPPING NON-ALLELE-SPECIFIC PRIMER AND ALLELE-SPECIFIC BLOCKER OLIGONUCLEOTIDES. Applicant: WILLIAM MARSH RICE UNIVERSITY. The sequence listing filed with the application follows.

SEQUENCE LISTING (49 sequences)

SEQ ID NO: 1 - DNA, 11 bp, Artificial Sequence
  Description of Artificial Sequence: Synthetic primer
agctgacctaa

SEQ ID NO: 2 - DNA, 11 bp, Artificial Sequence
  Description of Artificial Sequence: Synthetic oligonucleotide
  May be 3' C3 modified
acctaagcgat

SEQ ID NO: 3 - DNA, 22 bp, Artificial Sequence
  Description of Artificial Sequence: Synthetic primer
cagcctcatccaaaagaggaaa

SEQ ID NO: 4 - DNA, 27 bp, Artificial Sequence
  Description of Artificial Sequence: Synthetic oligonucleotide
  May be 3' C3 modified
aaaagaggaaacaggaccccagagctc

SEQ ID NO: 5 - DNA, 30 bp, Artificial Sequence
  Description of Artificial Sequence: Synthetic primer
tgtatatagacggtaaaataaacaccaaga

SEQ ID NO: 6 - DNA, 31 bp, Artificial Sequence
  Description of Artificial Sequence: Synthetic oligonucleotide
  May be 3' C3 modified
acaccaagacgtggtaaatatttacctggtc

SEQ ID NO: 7 - DNA, 29 bp, Artificial Sequence
  Description of Artificial Sequence: Synthetic primer
gagccttgtatatagacggtaaaataaac

SEQ ID NO: 8 - DNA, 36 bp, Artificial Sequence
  Description of Artificial Sequence: Synthetic oligonucleotide
  May be 3' C3 modified
cggtaaaataaacaccaagacgtggtaaatatttac

SEQ ID NO: 9 - DNA, 25 bp, Artificial Sequence
  Description of Artificial Sequence: Synthetic primer
tggagccttgtatatagacggtaaa

SEQ ID NO: 10 - DNA, 31 bp, Artificial Sequence
  Description of Artificial Sequence: Synthetic oligonucleotide
  May be 3' C3 modified
gacggtaaaataaacaccaagacgtggtaaa

SEQ ID NO: 11 - DNA, 23 bp, Artificial Sequence
  Description of Artificial Sequence: Synthetic primer
actggagccttgtatatagacgg

SEQ ID NO: 12 - DNA, 35 bp, Artificial Sequence
  Description of Artificial Sequence: Synthetic oligonucleotide
  May be 3' C3 modified
gtatatagacggtaaaataaacaccaagacgtggt

SEQ ID NO: 13 - DNA, 23 bp, Artificial Sequence
  Description of Artificial Sequence: Synthetic oligonucleotide
  May be 3' C3 modified
aaaagaggaaacaggaccccaga

SEQ ID NO: 14 - DNA, 24 bp, Artificial Sequence
  Description of Artificial Sequence: Synthetic oligonucleotide
  May be 3' C3 modified
aaaagaggaaacaggaccccagag

SEQ ID NO: 15 - DNA, 25 bp, Artificial Sequence
  Description of Artificial Sequence: Synthetic oligonucleotide
  May be 3' C3 modified
aaaagaggaaacaggaccccagagc

SEQ ID NO: 16 - DNA, 26 bp, Artificial Sequence
  Description of Artificial Sequence: Synthetic oligonucleotide
  May be 3' C3 modified
aaaagaggaaacaggaccccagagct

SEQ ID NO: 17 - DNA, 28 bp, Artificial Sequence
  Description of Artificial Sequence: Synthetic oligonucleotide
  May be 3' C3 modified
aaaagaggaaacaggaccccagagctcc

SEQ ID NO: 18 - DNA, 23 bp, Artificial Sequence
  Description of Artificial Sequence: Synthetic oligonucleotide
  May be 3' C3 modified
aaaagaggaaataggaccccaga

SEQ ID NO: 19 - DNA, 24 bp, Artificial Sequence
  Description of Artificial Sequence: Synthetic oligonucleotide
  May be 3' C3 modified
aaaagaggaaataggaccccagag

SEQ ID NO: 20 - DNA, 25 bp, Artificial Sequence
  Description of Artificial Sequence: Synthetic oligonucleotide
  May be 3' C3 modified
aaaagaggaaataggaccccagagc

SEQ ID NO: 21 - DNA, 26 bp, Artificial Sequence
  Description of Artificial Sequence: Synthetic oligonucleotide
  May be 3' C3 modified
aaaagaggaaataggaccccagagct

SEQ ID NO: 22 - DNA, 27 bp, Artificial Sequence
  Description of Artificial Sequence: Synthetic oligonucleotide
  May be 3' C3 modified
aaaagaggaaataggaccccagagctc

SEQ ID NO: 23 - DNA, 28 bp, Artificial Sequence
  Description of Artificial Sequence: Synthetic oligonucleotide
  May be 3' C3 modified
aaaagaggaaataggaccccagagctcc

SEQ ID NO: 24 - DNA, 35 bp, Artificial Sequence
  Description of Artificial Sequence: Synthetic oligonucleotide
acaccaagacgtggtaaatatttacctggtcaaaa

SEQ ID NO: 25 - DNA, 31 bp, Artificial Sequence
  Description of Artificial Sequence: Synthetic primer
cgatatggtttgtttcaaggtatgattttta

SEQ ID NO: 26 - DNA, 43 bp, Artificial Sequence
  Description of Artificial Sequence: Synthetic oligonucleotide
  May be 3' C3 modified
aaggtatgatttttaattaaaaattgttgttcacatttgaagg

SEQ ID NO: 27 - DNA, 25 bp, Artificial Sequence
  Description of Artificial Sequence: Synthetic primer
gtggtaaatatttacctggtccctg

SEQ ID NO: 28 - DNA, 35 bp, Artificial Sequence
  Description of Artificial Sequence: Synthetic oligonucleotide
  May be 3' C3 modified
ggtaaaataaacaccaagacgtggtaaatatttac

SEQ ID NO: 29 - DNA, 27 bp, Artificial Sequence
  Description of Artificial Sequence: Synthetic primer
tggagccttgtatatagacggtaaaat

SEQ ID NO: 30 - DNA, 31 bp, Artificial Sequence
  Description of Artificial Sequence: Synthetic oligonucleotide
  May be 3' C3 modified
accaggtaaatatttaccacgtcttggtgtt

SEQ ID NO: 31 - DNA, 27 bp, Artificial Sequence
  Description of Artificial Sequence: Synthetic primer
catcaacaacagggaccaggtaaatat

SEQ ID NO: 32 - DNA, 21 bp, Artificial Sequence
  Description of Artificial Sequence: Synthetic primer
ctcactctaaaccccagcatt

SEQ ID NO: 33 - DNA, 16 bp, Artificial Sequence
  Description of Artificial Sequence: Synthetic oligonucleotide
atcgcttaggtcagct

SEQ ID NO: 34 - DNA, 16 bp, Artificial Sequence
  Description of Artificial Sequence: Synthetic oligonucleotide
atcacttaggtcagct

SEQ ID NO: 35 - DNA, 44 bp, Artificial Sequence
  Description of Artificial Sequence: Synthetic oligonucleotide
agggagctctggggtcctatttcctcttttggatgaggctgtga

SEQ ID NO: 36 - DNA, 44 bp, Artificial Sequence
  Description of Artificial Sequence: Synthetic oligonucleotide
agggagctctggggtcctgtttcctcttttggatgaggctgtga

SEQ ID NO: 37 - DNA, 57 bp, Artificial Sequence
  Description of Artificial Sequence: Synthetic oligonucleotide
cagggaccaggtaaatatttaccacctcttggtgtttattttaccgtctatatacaa

SEQ ID NO: 38 - DNA, 57 bp, Artificial Sequence
  Description of Artificial Sequence: Synthetic oligonucleotide
cagggaccaggtaaatatttaccacgtcttggtgtttattttaccgtctatatacaa

SEQ ID NO: 39 - DNA, 67 bp, Artificial Sequence
  Description of Artificial Sequence: Synthetic oligonucleotide
cagggaccaggtaaatatttaccacctcttggtgtttattttaccgtctatatacaaggctccagtt

SEQ ID NO: 40 - DNA, 67 bp, Artificial Sequence
  Description of Artificial Sequence: Synthetic oligonucleotide
cagggaccaggtaaatatttaccacgtcttggtgtttattttaccgtctatatacaaggctccagtt

SEQ ID NO: 41 - DNA, 59 bp, Artificial Sequence
  Description of Artificial Sequence: Synthetic oligonucleotide
accttcaaatgtgaacaatttttaattaaaaatcataccttgaaacaaaccatatcgat

SEQ ID NO: 42 - DNA, 62 bp, Artificial Sequence
  Description of Artificial Sequence: Synthetic oligonucleotide
accttcaaatgtgaacaacaatttttaattaaaaatcataccttgaaacaaaccatatcgat

SEQ ID NO: 43 - DNA, 40 bp, Artificial Sequence
  Description of Artificial Sequence: Synthetic oligonucleotide
  May be 3' C3 modified
aaggtatgatttttaattaaaaattgttcacatttgaagg

SEQ ID NO: 44 - DNA, 47 bp, Artificial Sequence
  Description of Artificial Sequence: Synthetic oligonucleotide
acagggaccaggtaaatatttaccacctcttggtgtttattttaccg

SEQ ID NO: 45 - DNA, 47 bp, Artificial Sequence
  Description of Artificial Sequence: Synthetic oligonucleotide
acagggaccaggtaaatatttaccacgtcttggtgtttattttaccg

SEQ ID NO: 46 - DNA, 77 bp, Artificial Sequence
  Description of Artificial Sequence: Synthetic oligonucleotide
aacatcaacaacagggaccaggtaaatatttaccacctcttggtgtttattttaccgtctatatacaaggctccagt

SEQ ID NO: 47 - DNA, 77 bp, Artificial Sequence
  Description of Artificial Sequence: Synthetic oligonucleotide
aacatcaacaacagggaccaggtaaatatttaccacgtcttggtgtttattttaccgtctatatacaaggctccagt

SEQ ID NO: 48 - DNA, 77 bp, Artificial Sequence
  Description of Artificial Sequence: Synthetic oligonucleotide
actggagccttgtatatagacggtaaaataaacaccaagacgtggtaaatatttacctggtccctgttgttgatgtt

SEQ ID NO: 49 - DNA, 77 bp, Artificial Sequence
  Description of Artificial Sequence: Synthetic oligonucleotide
actggagccttgtatatagacggtaaaataaacaccaagaggtggtaaatatttacctggtccctgttgttgatgtt